European Patent Specification EP 4 003 989 B1, published December 27, 2023. Title: 6,7-dihydro-5H-pyrido[2,3-c]pyridazin-8-yl derivatives, pharmaceutical compositions containing them and their uses as pro-apoptotic agents. Applicant: Les Laboratoires Servier and Vernalis (R&D) Limited. The sequence listing filed with the application follows.

SEQUENCE LISTING (4 sequences)

SEQ ID NO: 1 - protein, 19 aa, Homo sapiens
AREIGAQLRRMADDLNAQY

SEQ ID NO: 2 - protein, 440 aa, Homo sapiens
MSPILGYWKIKGLVQPTRLLLEYLEEKYEEHLYERDEGDKWRNKKFELGLEFPNLPYYIDGDVKLTQSMAIIRYIADKHNMLGGCPKERAEISMLEGAVLDIRYGVSRIAYSKDFETLKVDFLSKLPEMLKMFEDRLCHKTYLNGDHVTHPDFMLYDALDVVLYMDPMCLDAFPKLVCFKKRIEAIPQIDKYLKSSKYIAWPLQGWQATFGGGDHPPKSDLIEGRGIPEFEFSQSNRELVVDFLSYKLSQKGYSWSQFSDVEENRTEAPEGTESEMETPSAINGNPSWHLADSPAVNGATGHSSSLDAREVIPMAAVKQALREAGDEFELRYRRAFSDLTSQLHITPGTAYQSFEQVVNELFRDGVNWGRIVAFFSFGGALCVESVDKEMQVLVSRIAAWMATYLNDHLEPWIQENGGWDTFVELYGNNAAAESRKGQER

SEQ ID NO: 3 - protein, 249 aa, Homo sapiens
MHHHHHHHHGATGSTAGSGTAGSTGASGASTGGTGATHHHHHHHHDDDDKSPMGSQSNRELVVDFLSYKLSQKGYSWSQFSDVEENRTEAPEGTESEMETPSAINGNPSWHLADSPAVNGATGHSSSLDAREVIPMAAVKQALREAGDEFELRYRRAFSDLTSQLHITPGTAYQSFEQVVNELFRDGVNWGRIVAFFSFGGALCVESVDKEMQVLVSRIAAWMATYLNDHLEPWIQENGGWDTFVELYG

SEQ ID NO: 4 - protein, 21 aa, Homo sapiens
QWAREIGAQLRRMADDLNAQY